European Patent Application EP 4 703 386 A1, published March 4, 2026. Title: 特异性结合CD276的抗体及其制备方法和应用. Applicant: 上海鑫湾生物科技有限公司. The sequence listing filed with the application follows.

SEQUENCE LISTING (330 sequences)

SEQ ID NO: 1 - DNA, 342 bp, synthetic construct
  source 1..342: mol_type = other DNA
caggtgacactgaaggaaagcggcggcggactggtgcagcctggaggatctctgagactgagttgtgctgcttctggcagcatctttaacatgtacgccatgggctggtacaggcaggcccctggaaaacagagagagctggtggcttccattacctctggaggctccacacactacgccgactccgtgaagggaagattcactatcagccgcgacaacgctaagaacacaatgtacctgcagatgaacagcctgaaacccgaagacaccgccgtgtactactgcagacagaacgatggaatggactactggggcaagggcaccctggtgacagtgagtagc

SEQ ID NO: 2 - protein, 114 aa, synthetic construct
QVTLKESGGGLVQPGGSLRLSCAASGSIFNMYAMGWYRQAPGKQRELVASITSGGSTHYADSVKGRFTISRDNAKNTMYLQMNSLKPEDTAVYYCRQNDGMDYWGKGTLVTVSS

SEQ ID NO: 3 - protein, 5 aa, synthetic construct
MYAMG

SEQ ID NO: 4 - protein, 16 aa, synthetic construct
SITSGGSTHYADSVKG

SEQ ID NO: 5 - protein, 6 aa, synthetic construct
NDGMDY

SEQ ID NO: 6 - DNA, 324 bp, synthetic construct
  source 1..324: mol_type = other DNA
caggctggactgacacagccaccaagcgtgagcgtggctcctggaaagacagccagaatcacatgcggcggcaacaacatcggctcaaagtccgtgcactggtaccagcagaagcccggacaggctcctgtggtggtgatctacgatgacagtgatagacctagcggcattcccgagcgctttagcggaagcaacagcggaaacaccgccaccctgactatcagccgcgtggaagctggcgatgaggctgatttctactgccaggtgtgggatagcagcagcgacagatacgtgttcgggaccggaaccaagctgacagtgctg

SEQ ID NO: 7 - protein, 108 aa, synthetic construct
QAGLTQPPSVSVAPGKTARITCGGNNIGSKSVHWYQQKPGQAPVVVIYDDSDRPSGIPERFSGSNSGNTATLTISRVEAGDEADFYCQVWDSSSDRYVFGTGTKLTVL

SEQ ID NO: 8 - protein, 11 aa, synthetic construct
GGNNIGSKSVH

SEQ ID NO: 9 - protein, 7 aa, synthetic construct
DDSDRPS

SEQ ID NO: 10 - protein, 11 aa, synthetic construct
QVWDSSSDRYV

SEQ ID NO: 11 - DNA, 360 bp, synthetic construct
  source 1..360: mol_type = other DNA
caggtgcagctggtgcagtcaggagctgaagtgaagaagcccggcgagtcactgagaatctcatgcaaaggcagcggctacagcttcacaagctactggatcagctgggtgagacagatgcccggcaaaggcctggagtggatgggaagaatcgaccccagtgacagctacaccaactactctcccagcttccagggccacgtgaccatctctgctgacaaaagcatcagcaccgcctacctgcagtggagcagcctgaaagccagcgacaccgctatgtattactgcgcccgccacgacgccagcggaggaggaccttctgattactggggccagggaaccctggtgaccgtgtcttct

SEQ ID NO: 12 - protein, 120 aa, synthetic construct
QVQLVQSGAEVKKPGESLRISCKGSGYSFTSYWISWVRQMPGKGLEWMGRIDPSDSYTNYSPSFQGHVTISADKSISTAYLQWSSLKASDTAMYYCARHDASGGGPSDYWGQGTLVTVSS

SEQ ID NO: 13 - protein, 5 aa, synthetic construct
SYWIS

SEQ ID NO: 14 - protein, 17 aa, synthetic construct
RIDPSDSYTNYSPSFQG

SEQ ID NO: 15 - protein, 11 aa, synthetic construct
HDASGGGPSDY

SEQ ID NO: 16 - DNA, 336 bp, synthetic construct
  source 1..336: mol_type = other DNA
cagtctgtgctgacccagccaccatccgtgtccgctgctcctggacagagagtgaccatcagctgcagcggctcctcatccaacatcggcgaccactacgtgtcctggtaccagcagctgcccggaactgctccaaaactgctgatctacgataataacaaaagaccaagtggcatccccgacagattcagcggctccaaaagcggaacctccgccacactgggcatcacaggactgcagacaggcgacgaggccgattactactgcggcacatgggacagcagcctgagtgtgcctaattgggtgttcggcggcggcacaaaggtgactgtgctg

SEQ ID NO: 17 - protein, 112 aa, synthetic construct
QSVLTQPPSVSAAPGQRVTISCSGSSSNIGDHYVSWYQQLPGTAPKLLIYDNNKRPSGIPDRFSGSKSGTSATLGITGLQTGDEADYYCGTWDSSLSVPNWVFGGGTKVTVL

SEQ ID NO: 18 - protein, 13 aa, synthetic construct
SGSSSNIGDHYVS

SEQ ID NO: 19 - protein, 7 aa, synthetic construct
DNNKRPS

SEQ ID NO: 20 - protein, 13 aa, synthetic construct
GTWDSSLSVPNWV

SEQ ID NO: 21 - DNA, 378 bp, synthetic construct
  source 1..378: mol_type = other DNA
cagatgcagctggtgcagagcggaggaggactggtgcagcctggaggaagtctgagactgagctgcgccgctagcggattcaccttcagcagctactggatgagctgggtgagacaggcccctggaaagggactggagtgggtggctaacattaaacaggacggaagcgagaaatactacgtggactctgtgaagggcagatttacaattagcagagacaacgccaagaacagcctgtatctgcagatgaacagcctgagggccgaagacaccgccgtgtattactgtgccaggagcccccactacgatttctggagaagggactactactacggaatggatgtgtggggccagggcaccctggtgacagtgtcttca

SEQ ID NO: 22 - protein, 126 aa, synthetic construct
QMQLVQSGGGLVQPGGSLRLSCAASGFTFSSYWMSWVRQAPGKGLEWVANIKQDGSEKYYVDSVKGRFTISRDNAKNSLYLQMNSLRAEDTAVYYCARSPHYDFWRRDYYYGMDVWGQGTLVTVSS

SEQ ID NO: 23 - protein, 5 aa, synthetic construct
SYWMS

SEQ ID NO: 24 - protein, 17 aa, synthetic construct
NIKQDGSEKYYVDSVKG

SEQ ID NO: 25 - protein, 17 aa, synthetic construct
SPHYDFWRRDYYYGMDV

SEQ ID NO: 26 - DNA, 330 bp, synthetic construct
  source 1..330: mol_type = other DNA
cagtctgtgctgacccagccaccatccgtgtccgctacaccaggacagaccgtgaccatcagctgcagcggaagcaccagcaacatcgccaccaactacgtgagctggtaccagcacctgcccggatctgctcctaaactgctgatctacgataacaacaagcgccccagcggcatccccgatagattctctggcagcaaaagcggaacctccgccaccctggacatcatcggactgcagacaggcgacgaagccgactactactgcggagtgtgggaccctagcctgacaacctacgtgttcggcaccggcacacagctgacagctctg

SEQ ID NO: 27 - protein, 110 aa, synthetic construct
QSVLTQPPSVSATPGQTVTISCSGSTSNIATNYVSWYQHLPGSAPKLLIYDNNKRPSGIPDRFSGSKSGTSATLDIIGLQTGDEADYYCGVWDPSLTTYVFGTGTQLTAL

SEQ ID NO: 28 - protein, 13 aa, synthetic construct
SGSTSNIATNYVS

SEQ ID NO: 29 - protein, 7 aa, synthetic construct
DNNKRPS

SEQ ID NO: 30 - protein, 11 aa, synthetic construct
GVWDPSLTTYV

SEQ ID NO: 31 - DNA, 363 bp, synthetic construct
  source 1..363: mol_type = other DNA
gaagtgcagctggtggagagcggaggaggagtggtgcagcctggaagaagcctgacactgagctgcgccgctagcggatttacctttaacggctatagcatgcactgggtgagacaggcccctggaaagggactggagtgggtggctgtgatgagcagcgatggaggaaacaagtactacgctgattccgtgaagggcagattcaccattagccgggacaacagcaagaacacactgtatctgcagatgaacggactgagacccgaggacaccgccgtgtattattgcgccagggccgtgagcagcggatggtctctgcctttcgacttctggggccacggcacactggtgactgtgtctagc

SEQ ID NO: 32 - protein, 121 aa, synthetic construct
EVQLVESGGGVVQPGRSLTLSCAASGFTFNGYSMHWVRQAPGKGLEWVAVMSSDGGNKYYADSVKGRFTISRDNSKNTLYLQMNGLRPEDTAVYYCARAVSSGWSLPFDFWGHGTLVTVSS

SEQ ID NO: 33 - protein, 5 aa, synthetic construct
GYSMH

SEQ ID NO: 34 - protein, 17 aa, synthetic construct
VMSSDGGNKYYADSVKG

SEQ ID NO: 35 - protein, 12 aa, synthetic construct
AVSSGWSLPFDF

SEQ ID NO: 36 - DNA, 321 bp, synthetic construct
  source 1..321: mol_type = other DNA
gatatcgtgatgacccagagccccagcagcctgtctacctctattggcgacagagtgaccattacctgcagagcctcccagggcatcagcaactttctggcctggtttcagcagaagcccggcaaggctcccaagtcactgatctacgccgcctccaggctgcagagtggagtgccttctaaattttccggctccggctctggcaccaacttcactctgactatcagctccctgcagcccgaagacttcgccacatactactgccagcagtacgactcctaccccctgaccttcggcggaggaacaaaggtggagatcaaa

SEQ ID NO: 37 - protein, 107 aa, synthetic construct
DIVMTQSPSSLSTSIGDRVTITCRASQGISNFLAWFQQKPGKAPKSLIYAASRLQSGVPSKFSGSGSGTNFTLTISSLQPEDFATYYCQQYDSYPLTFGGGTKVEIK

SEQ ID NO: 38 - protein, 11 aa, synthetic construct
RASQGISNFLA

SEQ ID NO: 39 - protein, 7 aa, synthetic construct
AASRLQS

SEQ ID NO: 40 - protein, 9 aa, synthetic construct
QQYDSYPLT

SEQ ID NO: 41 - DNA, 378 bp, synthetic construct
  source 1..378: mol_type = other DNA
caggtgcagctggtgcagtcaggagctgaagtgaagaagcccggcgcctcagtgagagtgagctgtaaaggaagcggctacaccttcacagaccaccacatgtactgggtgaggcaggccccaggacagggactggaatggatgggaagaatcaaccccaacaccggcgtgaccaattacgcccagaagttccagggcagagtgagcatgaccagagacaccagcatcaacacagtgtacctggagctgagaagcctgaagagcgacgacgccgctgtgtactactgcggaagagaccaggtggtgatggtgccaggggtgcctctggatctgggaatggacgtgtggggccagggaacaaccgtgacagtgagcagc

SEQ ID NO: 42 - protein, 126 aa, synthetic construct
QVQLVQSGAEVKKPGASVRVSCKGSGYTFTDHHMYWVRQAPGQGLEWMGRINPNTGVTNYAQKFQGRVSMTRDTSINTVYLELRSLKSDDAAVYYCGRDQVVMVPGVPLDLGMDVWGQGTTVTVSS

SEQ ID NO: 43 - protein, 5 aa, synthetic construct
DHHMY

SEQ ID NO: 44 - protein, 17 aa, synthetic construct
RINPNTGVTNYAQKFQG

SEQ ID NO: 45 - protein, 17 aa, synthetic construct
DQVVMVPGVPLDLGMDV

SEQ ID NO: 46 - DNA, 321 bp, synthetic construct
  source 1..321: mol_type = other DNA
aacatccagatgacccagagccccagcagcctgtcagcttctgtgggagacagagtgaccatcacctgcagagccagccagaccatcagcagatacctgaactggtaccagcagaaacccggcaaggccccaaaactgctgatttacgccgccagctccctgcagagcggagtgccttctagattcagcggaagcggcagcggcgctgatttcacactgactattaacaccctgcagcccgaggatttcgccacctactactgccagcagtcctaccgcaccccacagacttttggccagggcacaaaggtggaaatcaag

SEQ ID NO: 47 - protein, 107 aa, synthetic construct
NIQMTQSPSSLSASVGDRVTITCRASQTISRYLNWYQQKPGKAPKLLIYAASSLQSGVPSRFSGSGSGADFTLTINTLQPEDFATYYCQQSYRTPQTFGQGTKVEIK

SEQ ID NO: 48 - protein, 11 aa, synthetic construct
RASQTISRYLN

SEQ ID NO: 49 - protein, 7 aa, synthetic construct
AASSLQS

SEQ ID NO: 50 - protein, 9 aa, synthetic construct
QQSYRTPQT

SEQ ID NO: 51 - DNA, 357 bp, synthetic construct
  source 1..357: mol_type = other DNA
gaagtgcagctggtggagagcggaggaagaagcgtgcagtggggagagccactgagaatcagctgcaaggccagcgggttccagtttagcaactttgccatggcctggctgagacaggtgcccggaaaaggactggagtgggtgagcggagtgagcagtagcggaagcggaacctactacgccgacagtgtgaagggcagattcacaatcagcagagacaacgctaaaaacagcctgtacctgcagatgaacagcctgagggccgaggacaccgctgtgtattactgcgccagggagaccgtgaccacctcaggaatggacgtgtggggacagggaaccacagtgaccgtgagcagc

SEQ ID NO: 52 - protein, 119 aa, synthetic construct
EVQLVESGGRSVQWGEPLRISCKASGFQFSNFAMAWLRQVPGKGLEWVSGVSSSGSGTYYADSVKGRFTISRDNAKNSLYLQMNSLRAEDTAVYYCARETVTTSGMDVWGQGTTVTVSS

SEQ ID NO: 53 - protein, 5 aa, synthetic construct
NFAMA

SEQ ID NO: 54 - protein, 17 aa, synthetic construct
GVSSSGSGTYYADSVKG

SEQ ID NO: 55 - protein, 10 aa, synthetic construct
ETVTTSGMDV

SEQ ID NO: 56 - DNA, 329 bp, synthetic construct
  source 1..329: mol_type = other DNA
tcttacgtgctgacccagcctccttctgcctccggaactcctggacagagagtgaccatcagctgctctggctcctcctccaacatcggctccaacaccgtgaactggtaccagcagctgcccggaaccgctcctaagctgctgatttacagcaacaaccagagacccagcggcgtgccagataggttctccggaagcaaaagcggaacaagcgccagcctggccatctcaggactgcagtctgaggatgaagccgactactactgcgccgcctgggatgatagcctgaacggatgggtgtttggaggcggcacagagctgaccgtgct

SEQ ID NO: 57 - protein, 110 aa, synthetic construct
SYVLTQPPSASGTPGQRVTISCSGSSSNIGSNTVNWYQQLPGTAPKLLIYSNNQRPSGVPDRFSGSKSGTSASLAISGLQSEDEADYYCAAWDDSLNGWVFGGGTELTVL

SEQ ID NO: 58 - protein, 13 aa, synthetic construct
SGSSSNIGSNTVN

SEQ ID NO: 59 - protein, 7 aa, synthetic construct
SNNQRPS

SEQ ID NO: 60 - protein, 11 aa, synthetic construct
AAWDDSLNGWV

SEQ ID NO: 61 - DNA, 354 bp, synthetic construct
  source 1..354: mol_type = other DNA
caggtgcagctggtgcagtcaggaggaggactggtgcagccaggaggatcactgagactgagctgcgccgctagcggattcacattcagcaacagcgccatgagctggtacagacaggccccaggaaaggagagagagctggtggtgagaatctccggcggaacaggcaacctgttttacgccacctccgtggacagcgtgaagggaagattcaccatcagcagagacaacgccagaaacacagtgtacctgcacatgaatagcctgaagcccgaggacaccgccgtgtatttctgcaacgccgagaactttagagattactggggacagggcaccctggtgaccgtgtctagt

SEQ ID NO: 62 - protein, 118 aa, synthetic construct
QVQLVQSGGGLVQPGGSLRLSCAASGFTFSNSAMSWYRQAPGKERELVVRISGGTGNLFYATSVDSVKGRFTISRDNARNTVYLHMNSLKPEDTAVYFCNAENFRDYWGQGTLVTVSS

SEQ ID NO: 63 - protein, 5 aa, synthetic construct
NSAMS

SEQ ID NO: 64 - protein, 20 aa, synthetic construct
RISGGTGNLFYATSVDSVKG

SEQ ID NO: 65 - protein, 6 aa, synthetic construct
ENFRDY

SEQ ID NO: 66 - DNA, 309 bp, synthetic construct
  source 1..309: mol_type = other DNA
gatatccagctgacccagagccccagcaccctgtctgcttctgtgggagacagagtgaccattacctgcagagccagccagagcatcagcagctggctggcttggtaccagcagaagcccggaaaagccccaaaactgctgatctacaaaagctcaagcctggagagaggcgtgccctctagattcagcggaagcggaagcggcaccgaattcaccctgaccatcagcagcctgcagcccgatgattacgccacctactactgccagcaggacaactcatttggaggcggcacaaaggtggacatcaag

SEQ ID NO: 67 - protein, 103 aa, synthetic construct
DIQLTQSPSTLSASVGDRVTITCRASQSISSWLAWYQQKPGKAPKLLIYKSSSLERGVPSRFSGSGSGTEFTLTISSLQPDDYATYYCQQDNSFGGGTKVDIK

SEQ ID NO: 68 - protein, 11 aa, synthetic construct
RASQSISSWLA

SEQ ID NO: 69 - protein, 7 aa, synthetic construct
KSSSLER

SEQ ID NO: 70 - protein, 5 aa, synthetic construct
QQDNS

SEQ ID NO: 71 - DNA, 354 bp, synthetic construct
  source 1..354: mol_type = other DNA
gaagtgcagctggtgcagagcggagctgaggtgaagaagccaggagccagcgtgaaggtgagctgcaaggctagcgggtacacatttaccagctacggaatcagctgggtgagacaggccccaggacagggactggaatggatgggatggatcagcgcctacaacggaaatacaaactacgcccagaagctgcagggcagagtgacaatgaccacagacacaagcaccagcaccgcttacatggagctgagaagcctgaggagcgacgacacagccgtgtactactgcgccagagccccttattacggcggatatgactactggggccagggaaccatggtgaccgtgtcttcc

SEQ ID NO: 72 - protein, 118 aa, synthetic construct
EVQLVQSGAEVKKPGASVKVSCKASGYTFTSYGISWVRQAPGQGLEWMGWISAYNGNTNYAQKLQGRVTMTTDTSTSTAYMELRSLRSDDTAVYYCARAPYYGGYDYWGQGTMVTVSS

SEQ ID NO: 73 - protein, 5 aa, synthetic construct
SYGIS

SEQ ID NO: 74 - protein, 17 aa, synthetic construct
WISAYNGNTNYAQKLQG

SEQ ID NO: 75 - protein, 9 aa, synthetic construct
APYYGGYDY

SEQ ID NO: 76 - DNA, 327 bp, synthetic construct
  source 1..327: mol_type = other DNA
gaaacaaccctgacccagagccccggaaccctgtctctgagtcctggagacagagccaccctgagctgcagagctagccagtctgtgagaagcagctacctggcctggtaccagcagaagcccggacaggctccaagactggtgatctacggcgccagcaacagagccgctggaatccctgacagattttctggaagcggaagcggaacagacttcaccctgactatcagcggcctggaacccgaggactttgccgtgtattactgccaggagtacggctacagtctgcccaacacctttggccagggcacaaaactggagatcaaa

SEQ ID NO: 77 - protein, 109 aa, synthetic construct
ETTLTQSPGTLSLSPGDRATLSCRASQSVRSSYLAWYQQKPGQAPRLVIYGASNRAAGIPDRFSGSGSGTDFTLTISGLEPEDFAVYYCQEYGYSLPNTFGQGTKLEIK

SEQ ID NO: 78 - protein, 12 aa, synthetic construct
RASQSVRSSYLA

SEQ ID NO: 79 - protein, 7 aa, synthetic construct
GASNRAA

SEQ ID NO: 80 - protein, 10 aa, synthetic construct
QEYGYSLPNT

SEQ ID NO: 81 - DNA, 360 bp, synthetic construct
  source 1..360: mol_type = other DNA
gaagtgcagctggtggagacaggcggaggactggtgcagcctggaggatctctgagactgagctgcgccgctagcggatttaccttttccagctacggaatgacatgggtgagacagccacctggcaaaggactggagtgggtgagccacattagcggcagcggaaccaacacctactacgctgattctgtgaagggcagattcaccatcagcagagacaacagcaagaacaccctgtacctgcagatgaacaacctgggggccgaggacacagccgtgtattactgcgccaagctgaagtggggccatagcggatacggcgactactggggacagggaaccaccgtgaccgtgtctagc

SEQ ID NO: 82 - protein, 120 aa, synthetic construct
EVQLVETGGGLVQPGGSLRLSCAASGFTFSSYGMTWVRQPPGKGLEWVSHISGSGTNTYYADSVKGRFTISRDNSKNTLYLQMNNLGAEDTAVYYCAKLKWGHSGYGDYWGQGTTVTVSS

SEQ ID NO: 83 - protein, 5 aa, synthetic construct
SYGMT

SEQ ID NO: 84 - protein, 17 aa, synthetic construct
HISGSGTNTYYADSVKG

SEQ ID NO: 85 - protein, 11 aa, synthetic construct
LKWGHSGYGDY

SEQ ID NO: 86 - DNA, 324 bp, synthetic construct
  source 1..324: mol_type = other DNA
gaaatcgtgctgacccagagccccgctaccctgtctctgtctcctggagagagagccaccctgagctgcagagctagccagacaatcagcaggtacctggcctggtaccagcagaagcccggacaggctccaagactgctgatctacgacgccagcaacagagccacaggcattcccgctagattcagcggcagcggaagcgataccgacttcaccctgactatcagcagcatcgaaccagaggatttcgccgtgtactactgccaggagagaagcaactggccccaggtgacattcggacccggaacaaaactggagattaaa

SEQ ID NO: 87 - protein, 108 aa, synthetic construct
EIVLTQSPATLSLSPGERATLSCRASQTISRYLAWYQQKPGQAPRLLIYDASNRATGIPARFSGSGSDTDFTLTISSIEPEDFAVYYCQERSNWPQVTFGPGTKLEIK

SEQ ID NO: 88 - protein, 11 aa, synthetic construct
RASQTISRYLA

SEQ ID NO: 89 - protein, 7 aa, synthetic construct
DASNRAT

SEQ ID NO: 90 - protein, 10 aa, synthetic construct
QERSNWPQVT

SEQ ID NO: 91 - DNA, 375 bp, synthetic construct
  source 1..375: mol_type = other DNA
gaagtgcacctggtggagagcggaggaggactggtgcagcctggaggatcactgagactgagctgcgccgctagcggatttaccttttccagctacgccatgagctgggtgagacaggcccctggaaagggactggagtgggtgtctgccatttcaggcagcggaggcagcacctactacgctgattccgtgaagggccgctttaccatcagcagagacaacagcaagaacacactgtatctgcagatgaacagcctgagggccgaggacacagctgtgtactattgcgccagggtggggtactgcagtggcggatcttgctacgccggcggaatggatgtgtggggacagggaactaccgtgaccgtgtccagc

SEQ ID NO: 92 - protein, 125 aa, synthetic construct
EVHLVESGGGLVQPGGSLRLSCAASGFTFSSYAMSWVRQAPGKGLEWVSAISGSGGSTYYADSVKGRFTISRDNSKNTLYLQMNSLRAEDTAVYYCARVGYCSGGSCYAGGMDVWGQGTTVTVSS

SEQ ID NO: 93 - protein, 5 aa, synthetic construct
SYAMS

SEQ ID NO: 94 - protein, 17 aa, synthetic construct
AISGSGGSTYYADSVKG

SEQ ID NO: 95 - protein, 16 aa, synthetic construct
VGYCSGGSCYAGGMDV

SEQ ID NO: 96 - DNA, 324 bp, synthetic construct
  source 1..324: mol_type = other DNA
aacatccagatgacccagagccccagcagcctgtcagcttctgtgggagacagagtgaccatcacctgcagagccagccagagcatcagcagctacctgaactggtaccagcagaaacccggcaaggccccaaaactgctgatttacgccgccagctccctgcagagcggagtgccttctagattcagcggaagcggctccggcaccgatttcacactgactatttcaagcctgcagcccgaggatttcgccacctactactgccagcagtcctactccacaccaccatggaccttcggacagggcaccaaggtggagattaag

SEQ ID NO: 97 - protein, 108 aa, synthetic construct
NIQMTQSPSSLSASVGDRVTITCRASQSISSYLNWYQQKPGKAPKLLIYAASSLQSGVPSRFSGSGSGTDFTLTISSLQPEDFATYYCQQSYSTPPWTFGQGTKVEIK

SEQ ID NO: 98 - protein, 11 aa, synthetic construct
RASQSISSYLN

SEQ ID NO: 99 - protein, 7 aa, synthetic construct
AASSLQS

SEQ ID NO: 100 - protein, 10 aa, synthetic construct
QQSYSTPPWT

SEQ ID NO: 101 - protein, 366 aa, synthetic construct
GAAGTGCAGCTGGTGCAGAGCGGAGGAGGAGTGGTGCAGCCTGGAAGAAGCCTGAGACTGAGCTGCGCCGCTAGCGGATTTACCTTTTCCAGCTACGGAATGCACTGGGTGAGACAGGCCCCTGGAAAAGGGCTGGAGTGGGTGGCTGTGATCAGCTATGACGGCAGCAACAAATACTACGCTGATTCCGTGAAGGGCCGCTTTACCATCAGCAGAGACAACAGCAAGGACACACTGTATCTGCAGATGAACAGCCTGAGAGCCGAGGACACAGCCGTGTACTACTGCGCTAAGGACAAACTGATGGGGTGGCATAACTACGGCATGGACGTGTGGGGCCAGGGAACAACAGTGACCGTGAGCAGC

SEQ ID NO: 102 - protein, 122 aa, synthetic construct
EVQLVQSGGGVVQPGRSLRLSCAASGFTFSSYGMHWVRQAPGKGLEWVAVISYDGSNKYYADSVKGRFTISRDNSKDTLYLQMNSLRAEDTAVYYCAKDKLMGWHNYGMDVWGQGTTVTVSS

SEQ ID NO: 103 - protein, 5 aa, synthetic construct
SYGMH

SEQ ID NO: 104 - protein, 17 aa, synthetic construct
VISYDGSNKYYADSVKG

SEQ ID NO: 105 - protein, 13 aa, synthetic construct
DKLMGWHNYGMDV

SEQ ID NO: 106 - DNA, 321 bp, synthetic construct
  source 1..321: mol_type = other DNA
gctattcagctgacccagtccccttcctccctgtctgcttccgtgggagacagagtgaccattacctgtcgggcctcccagagtattaactcctacctgaactggtatcagcagaagcccggcaaagccccaaaagtgctgatctacgccgcctccaacctgcagagcggagtgccttctcgcttcagcggaagcggatccggaaccgatttcaccctgactatcagcagcctgcagcccgaagacttcgccacatactactgccagcagagctacagcaccccacctaccttcggccagggaacaaaactggagatcaaa

SEQ ID NO: 107 - protein, 107 aa, synthetic construct
AIQLTQSPSSLSASVGDRVTITCRASQSINSYLNWYQQKPGKAPKVLIYAASNLQSGVPSRFSGSGSGTDFTLTISSLQPEDFATYYCQQSYSTPPTFGQGTKLEIK

SEQ ID NO: 108 - protein, 11 aa, synthetic construct
RASQSINSYLN

SEQ ID NO: 109 - protein, 7 aa, synthetic construct
AASNLQS

SEQ ID NO: 110 - protein, 9 aa, synthetic construct
QQSYSTPPT

SEQ ID NO: 111 - DNA, 366 bp, synthetic construct
  source 1..366: mol_type = other DNA
gaagtgcagctggtgcagagcggaggaggactggtgaagcctggaggaagcctgagactgagctgcgctgctagcggatttacctttagtagacacagcatgaactgggtgagacaggcccctggcaaaggactggagtgggtgtcaagcatctcaagcaacgatgagcacatcatctacgccgattccgtgaagggcagattcaccatctcaagagacaacagcaagaacaccctgtacctggagatgaacagcctgagggccgaggacaccgctgtgtattactgcgcccgcgctagcagatacggaggatcatactacggcctggactactggggccagggaacactggtgaccgtgagtagc

SEQ ID NO: 112 - protein, 122 aa, synthetic construct
EVQLVQSGGGLVKPGGSLRLSCAASGFTFSRHSMNWVRQAPGKGLEWVSSISSNDEHIIYADSVKGRFTISRDNSKNTLYLEMNSLRAEDTAVYYCARASRYGGSYYGLDYWGQGTLVTVSS

SEQ ID NO: 113 - protein, 5 aa, synthetic construct
RHSMN

SEQ ID NO: 114 - protein, 17 aa, synthetic construct
SISSNDEHIIYADSVKG

SEQ ID NO: 115 - protein, 13 aa, synthetic construct
ASRYGGSYYGLDY

SEQ ID NO: 116 - DNA, 330 bp, synthetic construct
  source 1..330: mol_type = other DNA
cagacagtggtgacccaggagcctagcttcagcgtgagcccaggaggaaccgtgaccctgacatgcggactgacatcaggcagcgtgagcacaacctacttcccctcatggtaccagcagaccccaggccagccacctagaagactgatctataacaccaacaccagaagcagcggcgtgcccgatagattctccggaagcattgtgggcatcaaagccgccctgaccatcaccggagcccaggctgaagacgaaagcgactactactgcgccctgtacctgggcagcggaattgtggaattcggcggcggaacaaaactgaccgtgctg

SEQ ID NO: 117 - protein, 110 aa, synthetic construct
QTVVTQEPSFSVSPGGTVTLTCGLTSGSVSTTYFPSWYQQTPGQPPRRLIYNTNTRSSGVPDRFSGSIVGIKAALTITGAQAEDESDYYCALYLGSGIVEFGGGTKLTVL

SEQ ID NO: 118 - protein, 14 aa, synthetic construct
GLTSGSVSTTYFPS

SEQ ID NO: 119 - protein, 7 aa, synthetic construct
NTNTRSS

SEQ ID NO: 120 - protein, 10 aa, synthetic construct
ALYLGSGIVE

SEQ ID NO: 121 - DNA, 357 bp, synthetic construct
  source 1..357: mol_type = other DNA
caggtgcagctggtgcagtcaggaggaggagtggtgcagccaggaagaagcctgagactgagctgcgccgctagcggattcacattcagcagctacgccatgcattgggtgagacaggcccctggaaaaggactggagtgggtggctgtgattagctacgatggaagcaacaagtactacgccgacagcgtgaagggcagattcaccatcagcagagacaacagcaaaaacacactgtacctgcagatgaacagcctgagagccgaggacacaaccgtgtactactgcgccagagacagaagatactatagcagtatggacgtgtggggacagggaacaacagtgacagtgagcagc

SEQ ID NO: 122 - protein, 119 aa, synthetic construct
QVQLVQSGGGVVQPGRSLRLSCAASGFTFSSYAMHWVRQAPGKGLEWVAVISYDGSNKYYADSVKGRFTISRDNSKNTLYLQMNSLRAEDTTVYYCARDRRYYSSMDVWGQGTTVTVSS

SEQ ID NO: 123 - protein, 5 aa, synthetic construct
SYAMH

SEQ ID NO: 124 - protein, 17 aa, synthetic construct
VISYDGSNKYYADSVKG

SEQ ID NO: 125 - protein, 10 aa, synthetic construct
DRRYYSSMDV

SEQ ID NO: 126 - DNA, 330 bp, synthetic construct
  source 1..330: mol_type = other DNA
cagacagtggtgacccaggagcctagcttcagcgtgagcccaggaggaaccatcaccctgacctgcggactgagctccggatctgtgagcacctcctactaccccagctggtaccagcagaccccaggacaggctcctagaaccctgatctataacaccaataccagaagctccggcgtgcctgacagattcagcggaagcattctgggcaacaaggccgccctgaccatcacaggagcccaggctgatgacgaaagccactactactgcgccctgcacatggacagcggcagttgggtgttcggcggaggaacacagctgactgtgctg

SEQ ID NO: 127 - protein, 110 aa, synthetic construct
QTVVTQEPSFSVSPGGTITLTCGLSSGSVSTSYYPSWYQQTPGQAPRTLIYNTNTRSSGVPDRFSGSILGNKAALTITGAQADDESHYYCALHMDSGSWVFGGGTQLTVL

SEQ ID NO: 128 - protein, 14 aa, synthetic construct
GLSSGSVSTSYYPS

SEQ ID NO: 129 - protein, 7 aa, synthetic construct
NTNTRSS

SEQ ID NO: 130 - protein, 10 aa, synthetic construct
ALHMDSGSWV

SEQ ID NO: 131 - DNA, 345 bp, synthetic construct
  source 1..345: mol_type = other DNA
gaagtgcagctggtggagagcggaggaggactggtgcagcctggaggaagtctgagactgagctgcgccgctagcagaaacatcttcagattctacaccatgggatggtatagacaggcccctgagaagcagagagacctggtggctagaattaccagcgacggaaccaccaactacgccgacagcgtgaaaggccggttcaccatcagcagagacaacgccaagaacaccgtgtacctgcagatgaacagcctgaagcccgaggacaccgccgtgtattactgcaacaccgacctgcccctgaatacctactgggcccagggaaccctggtgacagtgtcaagc

SEQ ID NO: 132 - protein, 115 aa, synthetic construct
EVQLVESGGGLVQPGGSLRLSCAASRNIFRFYTMGWYRQAPEKQRDLVARITSDGTTNYADSVKGRFTISRDNAKNTVYLQMNSLKPEDTAVYYCNTDLPLNTYWAQGTLVTVSS

SEQ ID NO: 133 - protein, 5 aa, synthetic construct
FYTMG

SEQ ID NO: 134 - protein, 16 aa, synthetic construct
RITSDGTTNYADSVKG

SEQ ID NO: 135 - protein, 7 aa, synthetic construct
DLPLNTY

SEQ ID NO: 136 - DNA, 321 bp, synthetic construct
  source 1..321: mol_type = other DNA
gatatccagatgacccagagccccagcagcctgtctgcttctgtgggagacagagtgaccattacctgcagagctagccagagcattagcagctccctgaactggtaccagcacaagcccggcaaagccccaaagctgctgatctactccgcctccattctgcagagcggagtgccaagcagattctccggcagcggatcaggcacagactacaccctgactatcagcagcctgcagcctgaggatttcgccacctactcctgtcagcagtcctacaccacaccatataccttcggcctgggcaccaagctggagattaag

SEQ ID NO: 137 - protein, 107 aa, synthetic construct
DIQMTQSPSSLSASVGDRVTITCRASQSISSSLNWYQHKPGKAPKLLIYSASILQSGVPSRFSGSGSGTDYTLTISSLQPEDFATYSCQQSYTTPYTFGLGTKLEIK

SEQ ID NO: 138 - protein, 11 aa, synthetic construct
RASQSISSSLN

SEQ ID NO: 139 - protein, 7 aa, synthetic construct
SASILQS

SEQ ID NO: 140 - protein, 9 aa, synthetic construct
QQSYTTPYT

SEQ ID NO: 141 - protein, 8 aa, synthetic construct
GSIFNMYA

SEQ ID NO: 142 - protein, 7 aa, synthetic construct
ITSGGST

SEQ ID NO: 143 - protein, 8 aa, synthetic construct
RQNDGMDY

SEQ ID NO: 144 - protein, 7 aa, synthetic construct
GSIFNMY

SEQ ID NO: 145 - protein, 5 aa, synthetic construct
TSGGS

SEQ ID NO: 146 - protein, 6 aa, synthetic construct
NDGMDY

SEQ ID NO: 147 - protein, 6 aa, synthetic construct
NIGSKS

SEQ ID NO: 148 - skipped

SEQ ID NO: 149 - protein, 11 aa, synthetic construct
QVWDSSSDRYV

SEQ ID NO: 150 - protein, 11 aa, synthetic construct
GGNNIGSKSVH

SEQ ID NO: 151 - protein, 7 aa, synthetic construct
DDSDRPS

SEQ ID NO: 152 - protein, 11 aa, synthetic construct
QVWDSSSDRYV

SEQ ID NO: 153 - protein, 8 aa, synthetic construct
GYSFTSYW

SEQ ID NO: 154 - protein, 8 aa, synthetic construct
IDPSDSYT

SEQ ID NO: 155 - protein, 13 aa, synthetic construct
ARHDASGGGPSDY

SEQ ID NO: 156 - protein, 7 aa, synthetic construct
GYSFTSY

SEQ ID NO: 157 - protein, 6 aa, synthetic construct
DPSDSY

SEQ ID NO: 158 - protein, 11 aa, synthetic construct
HDASGGGPSDY

SEQ ID NO: 159 - protein, 8 aa, synthetic construct
SSNIGDHY

SEQ ID NO: 160 - skipped

SEQ ID NO: 161 - protein, 13 aa, synthetic construct
GTWDSSLSVPNWV

SEQ ID NO: 162 - protein, 13 aa, synthetic construct
SGSSSNIGDHYVS

SEQ ID NO: 163 - protein, 7 aa, synthetic construct
DNNKRPS

SEQ ID NO: 164 - protein, 13 aa, synthetic construct
GTWDSSLSVPNWV

SEQ ID NO: 165 - protein, 8 aa, synthetic construct
GFTFSSYW

SEQ ID NO: 166 - protein, 8 aa, synthetic construct
IKQDGSEK

SEQ ID NO: 167 - protein, 19 aa, synthetic construct
ARSPHYDFWRYYDRYGMDV

SEQ ID NO: 168 - protein, 7 aa, synthetic construct
GFTFSSY

SEQ ID NO: 169 - protein, 6 aa, synthetic construct
KQDGSE

SEQ ID NO: 170 - protein, 17 aa, synthetic construct
SPHYDFWRRDYYYGMDV

SEQ ID NO: 171 - protein, 8 aa, synthetic construct
TSNIATNY

SEQ ID NO: 172 - skipped

SEQ ID NO: 173 - protein, 11 aa, synthetic construct
GVWDPSLTTYV

SEQ ID NO: 174 - protein, 13 aa, synthetic construct
SGSTSNIATNYVS

SEQ ID NO: 175 - protein, 7 aa, synthetic construct
DNNKRPS

SEQ ID NO: 176 - protein, 11 aa, synthetic construct
GVWDPSLTTYV

SEQ ID NO: 177 - protein, 8 aa, synthetic construct
GFTFNGYS

SEQ ID NO: 178 - protein, 8 aa, synthetic construct
MSSDGGNK

SEQ ID NO: 179 - protein, 14 aa, synthetic construct
ARAVSSGSWLPFDF

SEQ ID NO: 180 - protein, 7 aa, synthetic construct
GFTFNGY

SEQ ID NO: 181 - protein, 6 aa, synthetic construct
SSDGGN

SEQ ID NO: 182 - protein, 12 aa, synthetic construct
AVSSGWSLPFDF

SEQ ID NO: 183 - protein, 6 aa, synthetic construct
QGISNF

SEQ ID NO: 184 - skipped

SEQ ID NO: 185 - protein, 9 aa, synthetic construct
QQYDSYPLT

SEQ ID NO: 186 - protein, 11 aa, synthetic construct
RASQGISNFLA

SEQ ID NO: 187 - protein, 7 aa, synthetic construct
AASRLQS

SEQ ID NO: 188 - protein, 9 aa, synthetic construct
QQYDSYPLT

SEQ ID NO: 189 - protein, 8 aa, synthetic construct
GYTFTDHH

SEQ ID NO: 190 - protein, 8 aa, synthetic construct
INPNTGVT

SEQ ID NO: 191 - protein, 19 aa, synthetic construct
GRDQVVMVPGDLPVLGMDV

SEQ ID NO: 192 - protein, 7 aa, synthetic construct
GYTFTDH

SEQ ID NO: 193 - protein, 6 aa, synthetic construct
NPNTGV

SEQ ID NO: 194 - protein, 17 aa, synthetic construct
DQVVMVPGVPLDLGMDV

SEQ ID NO: 195 - protein, 6 aa, synthetic construct
QTISRY

SEQ ID NO: 196 - skipped

SEQ ID NO: 197 - protein, 9 aa, synthetic construct
QQSYRTPQT

SEQ ID NO: 198 - protein, 11 aa, synthetic construct
RASQTISRYLN

SEQ ID NO: 199 - protein, 7 aa, synthetic construct
AASSLQS

SEQ ID NO: 200 - protein, 9 aa, synthetic construct
QQSYRTPQT

SEQ ID NO: 201 - protein, 8 aa, synthetic construct
GFQFSNFA

SEQ ID NO: 202 - protein, 8 aa, synthetic construct
VSSSGSGT

SEQ ID NO: 203 - protein, 12 aa, synthetic construct
ARETVTTSGMDV

SEQ ID NO: 204 - protein, 7 aa, synthetic construct
GFQFSNF

SEQ ID NO: 205 - protein, 6 aa, synthetic construct
SSSGSG

SEQ ID NO: 206 - protein, 10 aa, synthetic construct
ETVTTSGMDV

SEQ ID NO: 207 - protein, 8 aa, synthetic construct
SSNIGSNT

SEQ ID NO: 208 - skipped

SEQ ID NO: 209 - protein, 11 aa, synthetic construct
AAWDDSLNGWV

SEQ ID NO: 210 - protein, 13 aa, synthetic construct
SGSSSNIGSNTVN

SEQ ID NO: 211 - protein, 7 aa, synthetic construct
SNNQRPS

SEQ ID NO: 212 - protein, 11 aa, synthetic construct
AAWDDSLNGWV

SEQ ID NO: 213 - protein, 8 aa, synthetic construct
GFTFSNSA

SEQ ID NO: 214 - protein, 8 aa, synthetic construct
ISGGTGNL

SEQ ID NO: 215 - protein, 8 aa, synthetic construct
NAENFRDY

SEQ ID NO: 216 - protein, 7 aa, synthetic construct
GFTFSNS

SEQ ID NO: 217 - protein, 6 aa, synthetic construct
SGGTGN

SEQ ID NO: 218 - protein, 6 aa, synthetic construct
ENFRDY

SEQ ID NO: 219 - protein, 6 aa, synthetic construct
QSISSW

SEQ ID NO: 220 - skipped

SEQ ID NO: 221 - protein, 5 aa, synthetic construct
QQDNS

SEQ ID NO: 222 - protein, 11 aa, synthetic construct
RASQSISSWLA

SEQ ID NO: 223 - protein, 7 aa, synthetic construct
KSSSLER

SEQ ID NO: 224 - protein, 5 aa, synthetic construct
QQDNS

SEQ ID NO: 225 - protein, 8 aa, synthetic construct
GYTFTSYG

SEQ ID NO: 226 - protein, 8 aa, synthetic construct
ISAYNGNT

SEQ ID NO: 227 - protein, 11 aa, synthetic construct
ARAPYYGGYDY

SEQ ID NO: 228 - protein, 7 aa, synthetic construct
GYTFTSY

SEQ ID NO: 229 - protein, 6 aa, synthetic construct
SAYNGN

SEQ ID NO: 230 - protein, 9 aa, synthetic construct
APYYGGYDY

SEQ ID NO: 231 - protein, 7 aa, synthetic construct
QSVRSSY

SEQ ID NO: 232 - skipped

SEQ ID NO: 233 - protein, 10 aa, synthetic construct
QEYGYSLPNT

SEQ ID NO: 234 - protein, 12 aa, synthetic construct
RASQSVRSSYLA

SEQ ID NO: 235 - protein, 7 aa, synthetic construct
GASNRAA

SEQ ID NO: 236 - protein, 10 aa, synthetic construct
QEYGYSLPNT

SEQ ID NO: 237 - protein, 8 aa, synthetic construct
GFTFSSYG

SEQ ID NO: 238 - protein, 8 aa, synthetic construct
ISGSGTNT

SEQ ID NO: 239 - protein, 13 aa, synthetic construct
AKLKWGHSGYGDY

SEQ ID NO: 240 - protein, 7 aa, synthetic construct
GFTFSSY

SEQ ID NO: 241 - protein, 6 aa, synthetic construct
SGSGTN

SEQ ID NO: 242 - protein, 11 aa, synthetic construct
LKWGHSGYGDY

SEQ ID NO: 243 - protein, 6 aa, synthetic construct
QTISRY

SEQ ID NO: 244 - skipped

SEQ ID NO: 245 - protein, 10 aa, synthetic construct
QERSNWPQVT

SEQ ID NO: 246 - protein, 11 aa, synthetic construct
RASQTISRYLA

SEQ ID NO: 247 - protein, 7 aa, synthetic construct
DASNRAT

SEQ ID NO: 248 - protein, 10 aa, synthetic construct
QERSNWPQVT

SEQ ID NO: 249 - protein, 8 aa, synthetic construct
GFTFSSYA

SEQ ID NO: 250 - protein, 8 aa, synthetic construct
ISGSGGST

SEQ ID NO: 251 - protein, 18 aa, synthetic construct
ARVGYCSGGAYCSGGMDV

SEQ ID NO: 252 - protein, 7 aa, synthetic construct
GFTFSSY

SEQ ID NO: 253 - protein, 6 aa, synthetic construct
SGSGGS

SEQ ID NO: 254 - protein, 16 aa, synthetic construct
VGYCSGGSCYAGGMDV

SEQ ID NO: 255 - protein, 6 aa, synthetic construct
QSISSY

SEQ ID NO: 256 - skipped

SEQ ID NO: 257 - protein, 10 aa, synthetic construct
QQSYSTPPWT

SEQ ID NO: 258 - protein, 11 aa, synthetic construct
RASQSISSYLN

SEQ ID NO: 259 - protein, 7 aa, synthetic construct
AASSLQS

SEQ ID NO: 260 - protein, 10 aa, synthetic construct
QQSYSTPPWT

SEQ ID NO: 261 - protein, 8 aa, synthetic construct
GFTFSSYG

SEQ ID NO: 262 - protein, 8 aa, synthetic construct
ISYDGSNK

SEQ ID NO: 263 - protein, 15 aa, synthetic construct
AKDKLMGWNHYGMDV

SEQ ID NO: 264 - protein, 7 aa, synthetic construct
GFTFSSY

SEQ ID NO: 265 - protein, 6 aa, synthetic construct
SYDGSN

SEQ ID NO: 266 - protein, 13 aa, synthetic construct
DKLMGWHNYGMDV

SEQ ID NO: 267 - protein, 6 aa, synthetic construct
QSINSY

SEQ ID NO: 268 - skipped

SEQ ID NO: 269 - protein, 9 aa, synthetic construct
QQSYSTPPT

SEQ ID NO: 270 - protein, 11 aa, synthetic construct
RASQSINSYLN

SEQ ID NO: 271 - protein, 7 aa, synthetic construct
AASNLQS

SEQ ID NO: 272 - protein, 9 aa, synthetic construct
QQSYSTPPT

SEQ ID NO: 273 - protein, 8 aa, synthetic construct
GFTFSRHS

SEQ ID NO: 274 - protein, 8 aa, synthetic construct
ISSNDEHI

SEQ ID NO: 275 - protein, 15 aa, synthetic construct
ARASRYGGYSYGLDY

SEQ ID NO: 276 - protein, 7 aa, synthetic construct
GFTFSRH

SEQ ID NO: 277 - protein, 6 aa, synthetic construct
SSNDEH

SEQ ID NO: 278 - protein, 13 aa, synthetic construct
ASRYGGSYYGLDY

SEQ ID NO: 279 - protein, 9 aa, synthetic construct
SGSVSTTYF

SEQ ID NO: 280 - skipped

SEQ ID NO: 281 - protein, 10 aa, synthetic construct
ALYLGSGIVE

SEQ ID NO: 282 - protein, 14 aa, synthetic construct
GLTSGSVSTTYFPS

SEQ ID NO: 283 - protein, 7 aa, synthetic construct
NTNTRSS

SEQ ID NO: 284 - protein, 10 aa, synthetic construct
ALYLGSGIVE

SEQ ID NO: 285 - protein, 8 aa, synthetic construct
GFTFSSYA

SEQ ID NO: 286 - protein, 8 aa, synthetic construct
ISYDGSNK

SEQ ID NO: 287 - protein, 12 aa, synthetic construct
ARDRRYYSSMDV

SEQ ID NO: 288 - protein, 7 aa, synthetic construct
GFTFSSY

SEQ ID NO: 289 - protein, 6 aa, synthetic construct
SYDGSN

SEQ ID NO: 290 - protein, 10 aa, synthetic construct
DRRYYSSMDV

SEQ ID NO: 291 - protein, 9 aa, synthetic construct
SGSVSTSYY

SEQ ID NO: 292 - skipped

SEQ ID NO: 293 - protein, 10 aa, synthetic construct
ALHMDSGSWV

SEQ ID NO: 294 - protein, 14 aa, synthetic construct
GLSSGSVSTSYYPS

SEQ ID NO: 295 - protein, 7 aa, synthetic construct
NTNTRSS

SEQ ID NO: 296 - protein, 10 aa, synthetic construct
ALHMDSGSWV

SEQ ID NO: 297 - protein, 8 aa, synthetic construct
RNIFRFYT

SEQ ID NO: 298 - protein, 7 aa, synthetic construct
ITSDGTT

SEQ ID NO: 299 - protein, 9 aa, synthetic construct
NTDLPLNTY

SEQ ID NO: 300 - protein, 7 aa, synthetic construct
RNIFRFY

SEQ ID NO: 301 - protein, 5 aa, synthetic construct
TSDGT

SEQ ID NO: 302 - protein, 7 aa, synthetic construct
DLPLNTY

SEQ ID NO: 303 - protein, 6 aa, synthetic construct
QSISSS

SEQ ID NO: 304 - skipped

SEQ ID NO: 305 - protein, 9 aa, synthetic construct
QQSYTTPYT

SEQ ID NO: 306 - protein, 11 aa, synthetic construct
RASQSISSSLN

SEQ ID NO: 307 - protein, 7 aa, synthetic construct
SASILQS

SEQ ID NO: 308 - protein, 9 aa, synthetic construct
QQSYTTPYT

SEQ ID NO: 309 - protein, 242 aa, synthetic construct
QVQLVQSGAEVKKPGASVKVSCKASGYTFTRYTMHWVRQAPGQGLEWMGYINPSRGYTNYNQKFKDRVTITADKSTSTAYMELSSLRSEDTAVYYCARYYDDHYCLDYWGQGTTVTVSSGGGGSGGGGSGGGGSGSEIVLTQSPATLSLSPGERATLSCSASSSVSYMNWYQQKPGKAPKRLIYDTSKLASGVPSRFSGSGSGTDFTLTINSLEAEDAATYYCQQWSSNPFTFGQGTKVEIK

SEQ ID NO: 310 - protein, 243 aa, synthetic construct
QVQLVQSGAEVKKPGASVKVSCKASGYTFTRYTMHWVRQAPGQGLEWMGYINPSRGYTNYNQKFKDRVTITADKSTSTAYMELSSLRSEDTAVYYCARYYDDHYCLDYWGQGTTVTVSSGGGGSGGGGSGGGGSGSEIVLTQSPATLSLSPGERATLSCSASSSVSYMNWYQQKPGKAPKRLIYDTSKLASGVPSRFSGSGSGTDFTLTINSLEAEDAATYYCQQWSSNPFTFGQGTKVEIKR

SEQ ID NO: 311 - DNA, 1503 bp, synthetic construct
  source 1..1503: mol_type = other DNA
atgggatggtcatgtatcatcctgttcctagtagcaactgcaaccggtcaggctggactgacacagccaccaagcgtgagcgtggctcctggaaagacagccagaatcacatgcggcggcaacaacatcggctcaaagtccgtgcactggtaccagcagaagcccggacaggctcctgtggtggtgatctacgatgacagtgatagacctagcggcattcccgagcgctttagcggaagcaacagcggaaacaccgccaccctgactatcagccgcgtggaagctggcgatgaggctgatttctactgccaggtgtgggatagcagcagcgacagatacgtgttcgggaccggaaccaagctgacagtgctgggcggaggaggctccggaggtggaggaagcggcggaggcggcagccaggtgacactgaaggaaagcggcggcggactggtgcagcctggaggatctctgagactgagttgtgctgcttctggcagcatctttaacatgtacgccatgggctggtacaggcaggcccctggaaaacagagagagctggtggcttccattacctctggaggctccacacactacgccgactccgtgaagggaagattcactatcagccgcgacaacgctaagaacacaatgtacctgcagatgaacagcctgaaacccgaagacaccgccgtgtactactgcagacagaacgatggaatggactactggggcaagggcaccctggtgacagtgagtagcggagggggcggatcccaggtccaactcgttcaaagcggagctgaggtgaagaagcctggcgcctccgtgaaggtgtcctgtaaggcctccggctacacctttaccaggtacacaatgcactgggtcaggcaggctcctggccagggcctggagtggatgggctacatcaatcctagcaggggctacacaaattacaaccagaagtttaaggacagagtgacaatcacagccgataagagcaccagcactgcttatatggaactgtccagcctgaggtccgaggacaccgccgtgtactactgtgccaggtactacgatgaccactactgcctggattactggggccagggcaccaccgtgacagtgagcagcggcggcggcggaagcggaggcggaggaagcggcggaggaggatctggcagcgagatcgtgctgacccagagccctgccaccctgagcctgagccctggcgagagggccaccctgtcctgctccgcttccagcagcgtgtcctacatgaactggtatcaacaaaagcctggcaaagctcctaagagactgatctacgacacctccaagctggcctccggcgtgccatccagattctccggctccggcagcggcaccgattttaccctgaccatcaacagcctcgaagccgaggacgccgccacatactactgccagcagtggagctccaacccttttaccttcggccagggcacaaaggtggagatcaagagg

SEQ ID NO: 312 - protein, 501 aa, synthetic construct
MGWSCIILFLVATATGQAGLTQPPSVSVAPGKTARITCGGNNIGSKSVHWYQQKPGQAPVVVIYDDSDRPSGIPERFSGSNSGNTATLTISRVEAGDEADFYCQVWDSSSDRYVFGTGTKLTVLGGGGSGGGGSGGGGSQVTLKESGGGLVQPGGSLRLSCAASGSIFNMYAMGWYRQAPGKQRELVASITSGGSTHYADSVKGRFTISRDNAKNTMYLQMNSLKPEDTAVYYCRQNDGMDYWGKGTLVTVSSGGGGSQVQLVQSGAEVKKPGASVKVSCKASGYTFTRYTMHWVRQAPGQGLEWMGYINPSRGYTNYNQKFKDRVTITADKSTSTAYMELSSLRSEDTAVYYCARYYDDHYCLDYWGQGTTVTVSSGGGGSGGGGSGGGGSGSEIVLTQSPATLSLSPGERATLSCSASSSVSYMNWYQQKPGKAPKRLIYDTSKLASGVPSRFSGSGSGTDFTLTINSLEAEDAATYYCQQWSSNPFTFGQGTKVEIKR

SEQ ID NO: 313 - DNA, 1521 bp, synthetic construct
  source 1..1521: mol_type = other DNA
atgggatggtcatgtatcatcctgttcctagtagcaactgcaaccggtgatatcgtgatgacccagagccccagcagcctgtctacctctattggcgacagagtgaccattacctgcagagcctcccagggcatcagcaactttctggcctggtttcagcagaagcccggcaaggctcccaagtcactgatctacgccgcctccaggctgcagagtggagtgccttctaaattttccggctccggctctggcaccaacttcactctgactatcagctccctgcagcccgaagacttcgccacatactactgccagcagtacgactcctaccccctgaccttcggcggaggaacaaaggtggagatcaaaggcggaggaggctccggaggtggaggaagcggcggaggcggcagcgaagtgcagctggtggagagcggaggaggagtggtgcagcctggaagaagcctgacactgagctgcgccgctagcggatttacctttaacggctatagcatgcactgggtgagacaggcccctggaaagggactggagtgggtggctgtgatgagcagcgatggaggaaacaagtactacgctgattccgtgaagggcagattcaccattagccgggacaacagcaagaacacactgtatctgcagatgaacggactgagacccgaggacaccgccgtgtattattgcgccagggccgtgagcagcggatggtctctgcctttcgacttctggggccacggcacactggtgactgtgtctagcggagggggcggatcccaggtccaactcgttcaaagcggagctgaggtgaagaagcctggcgcctccgtgaaggtgtcctgtaaggcctccggctacacctttaccaggtacacaatgcactgggtcaggcaggctcctggccagggcctggagtggatgggctacatcaatcctagcaggggctacacaaattacaaccagaagtttaaggacagagtgacaatcacagccgataagagcaccagcactgcttatatggaactgtccagcctgaggtccgaggacaccgccgtgtactactgtgccaggtactacgatgaccactactgcctggattactggggccagggcaccaccgtgacagtgagcagcggcggcggcggaagcggaggcggaggaagcggcggaggaggatctggcagcgagatcgtgctgacccagagccctgccaccctgagcctgagccctggcgagagggccaccctgtcctgctccgcttccagcagcgtgtcctacatgaactggtatcaacaaaagcctggcaaagctcctaagagactgatctacgacacctccaagctggcctccggcgtgccatccagattctccggctccggcagcggcaccgattttaccctgaccatcaacagcctcgaagccgaggacgccgccacatactactgccagcagtggagctccaacccttttaccttcggccagggcacaaaggtggagatcaagagg

SEQ ID NO: 314 - protein, 507 aa, synthetic construct
MGWSCIILFLVATATGDIVMTQSPSSLSTSIGDRVTITCRASQGISNFLAWFQQKPGKAPKSLIYAASRLQSGVPSKFSGSGSGTNFTLTISSLQPEDFATYYCQQYDSYPLTFGGGTKVEIKGGGGSGGGGSGGGGSEVQLVESGGGVVQPGRSLTLSCAASGFTFNGYSMHWVRQAPGKGLEWVAVMSSDGGNKYYADSVKGRFTISRDNSKNTLYLQMNGLRPEDTAVYYCARAVSSGWSLPFDFWGHGTLVTVSSGGGGSQVQLVQSGAEVKKPGASVKVSCKASGYTFTRYTMHWVRQAPGQGLEWMGYINPSRGYTNYNQKFKDRVTITADKSTSTAYMELSSLRSEDTAVYYCARYYDDHYCLDYWGQGTTVTVSSGGGGSGGGGSGGGGSGSEIVLTQSPATLSLSPGERATLSCSASSSVSYMNWYQQKPGKAPKRLIYDTSKLASGVPSRFSGSGSGTDFTLTINSLEAEDAATYYCQQWSSNPFTFGQGTKVEIKR

SEQ ID NO: 315 - DNA, 1536 bp, synthetic construct
  source 1..1536: mol_type = other DNA
atgggatggtcatgtatcatcctgttcctagtagcaactgcaaccggtaacatccagatgacccagagccccagcagcctgtcagcttctgtgggagacagagtgaccatcacctgcagagccagccagaccatcagcagatacctgaactggtaccagcagaaacccggcaaggccccaaaactgctgatttacgccgccagctccctgcagagcggagtgccttctagattcagcggaagcggcagcggcgctgatttcacactgactattaacaccctgcagcccgaggatttcgccacctactactgccagcagtcctaccgcaccccacagacttttggccagggcacaaaggtggaaatcaagggcggaggaggctccggaggtggaggaagcggcggaggcggcagccaggtgcagctggtgcagtcaggagctgaagtgaagaagcccggcgcctcagtgagagtgagctgtaaaggaagcggctacaccttcacagaccaccacatgtactgggtgaggcaggccccaggacagggactggaatggatgggaagaatcaaccccaacaccggcgtgaccaattacgcccagaagttccagggcagagtgagcatgaccagagacaccagcatcaacacagtgtacctggagctgagaagcctgaagagcgacgacgccgctgtgtactactgcggaagagaccaggtggtgatggtgccaggggtgcctctggatctgggaatggacgtgtggggccagggaacaaccgtgacagtgagcagcggagggggcggatcccaggtccaactcgttcaaagcggagctgaggtgaagaagcctggcgcctccgtgaaggtgtcctgtaaggcctccggctacacctttaccaggtacacaatgcactgggtcaggcaggctcctggccagggcctggagtggatgggctacatcaatcctagcaggggctacacaaattacaaccagaagtttaaggacagagtgacaatcacagccgataagagcaccagcactgcttatatggaactgtccagcctgaggtccgaggacaccgccgtgtactactgtgccaggtactacgatgaccactactgcctggattactggggccagggcaccaccgtgacagtgagcagcggcggcggcggaagcggaggcggaggaagcggcggaggaggatctggcagcgagatcgtgctgacccagagccctgccaccctgagcctgagccctggcgagagggccaccctgtcctgctccgcttccagcagcgtgtcctacatgaactggtatcaacaaaagcctggcaaagctcctaagagactgatctacgacacctccaagctggcctccggcgtgccatccagattctccggctccggcagcggcaccgattttaccctgaccatcaacagcctcgaagccgaggacgccgccacatactactgccagcagtggagctccaacccttttaccttcggccagggcacaaaggtggagatcaagagg

SEQ ID NO: 316 - protein, 512 aa, synthetic construct
MGWSCIILFLVATATGNIQMTQSPSSLSASVGDRVTITCRASQTISRYLNWYQQKPGKAPKLLIYAASSLQSGVPSRFSGSGSGADFTLTINTLQPEDFATYYCQQSYRTPQTFGQGTKVEIKGGGGSGGGGSGGGGSQVQLVQSGAEVKKPGASVRVSCKGSGYTFTDHHMYWVRQAPGQGLEWMGRINPNTGVTNYAQKFQGRVSMTRDTSINTVYLELRSLKSDDAAVYYCGRDQVVMVPGVPLDLGMDVWGQGTTVTVSSGGGGSQVQLVQSGAEVKKPGASVKVSCKASGYTFTRYTMHWVRQAPGQGLEWMGYINPSRGYTNYNQKFKDRVTITADKSTSTAYMELSSLRSEDTAVYYCARYYDDHYCLDYWGQGTTVTVSSGGGGSGGGGSGGGGSGSEIVLTQSPATLSLSPGERATLSCSASSSVSYMNWYQQKPGKAPKRLIYDTSKLASGVPSRFSGSGSGTDFTLTINSLEAEDAATYYCQQWSSNPFTFGQGTKVEIKR

SEQ ID NO: 317 - DNA, 1533 bp, synthetic construct
  source 1..1533: mol_type = other DNA
atgggatggtcatgtatcatcctgttcctagtagcaactgcaaccggtcagacagtggtgacccaggagcctagcttcagcgtgagcccaggaggaaccgtgaccctgacatgcggactgacatcaggcagcgtgagcacaacctacttcccctcatggtaccagcagaccccaggccagccacctagaagactgatctataacaccaacaccagaagcagcggcgtgcccgatagattctccggaagcattgtgggcatcaaagccgccctgaccatcaccggagcccaggctgaagacgaaagcgactactactgcgccctgtacctgggcagcggaattgtggaattcggcggcggaacaaaactgaccgtgctgggcggaggaggctccggaggtggaggaagcggcggaggcggcagcgaagtgcagctggtgcagagcggaggaggactggtgaagcctggaggaagcctgagactgagctgcgctgctagcggatttacctttagtagacacagcatgaactgggtgagacaggcccctggcaaaggactggagtgggtgtcaagcatctcaagcaacgatgagcacatcatctacgccgattccgtgaagggcagattcaccatctcaagagacaacagcaagaacaccctgtacctggagatgaacagcctgagggccgaggacaccgctgtgtattactgcgcccgcgctagcagatacggaggatcatactacggcctggactactggggccagggaacactggtgaccgtgagtagcggagggggcggatcccaggtgcagctggtgcagtccggcgccgaggtgaagaagcctggcgcctccgtgaaggtgtcctgtaaggcctccggctacacctttaccaggtacacaatgcactgggtcaggcaggctcctggccagggcctggagtggatgggctacatcaatcctagcaggggctacacaaattacaaccagaagtttaaggacagagtgacaatcacagccgataagagcaccagcactgcttatatggaactgtccagcctgaggtccgaggacaccgccgtgtactactgtgccaggtactacgatgaccactactgcctggattactggggccagggcaccaccgtgacagtgagcagcggcggcggcggaagcggaggcggaggaagcggcggaggaggatctggcagcgagatcgtgctgacccagagccctgccaccctgagcctgagccctggcgagagggccaccctgtcctgctccgcttccagcagcgtgtcctacatgaactggtatcaacaaaagcctggcaaagctcctaagagactgatctacgacacctccaagctggcctccggcgtgccatccagattctccggctccggcagcggcaccgattttaccctgaccatcaacagcctcgaagccgaggacgccgccacatactactgccagcagtggagctccaacccttttaccttcggccagggcacaaaggtggagatcaagagg

SEQ ID NO: 318 - protein, 511 aa, synthetic construct
MGWSCIILFLVATATGQTVVTQEPSFSVSPGGTVTLTCGLTSGSVSTTYFPSWYQQTPGQPPRRLIYNTNTRSSGVPDRFSGSIVGIKAALTITGAQAEDESDYYCALYLGSGIVEFGGGTKLTVLGGGGSGGGGSGGGGSEVQLVQSGGGLVKPGGSLRLSCAASGFTFSRHSMNWVRQAPGKGLEWVSSISSNDEHIIYADSVKGRFTISRDNSKNTLYLEMNSLRAEDTAVYYCARASRYGGSYYGLDYWGQGTLVTVSSGGGGSQVQLVQSGAEVKKPGASVKVSCKASGYTFTRYTMHWVRQAPGQGLEWMGYINPSRGYTNYNQKFKDRVTITADKSTSTAYMELSSLRSEDTAVYYCARYYDDHYCLDYWGQGTTVTVSSGGGGSGGGGSGGGGSGSEIVLTQSPATLSLSPGERATLSCSASSSVSYMNWYQQKPGKAPKRLIYDTSKLASGVPSRFSGSGSGTDFTLTINSLEAEDAATYYCQQWSSNPFTFGQGTKVEIKR

SEQ ID NO: 319 - DNA, 2207 bp, synthetic construct
  source 1..2207: mol_type = other DNA
gacattgattattgactagttattaatagtaatcaattacggggtcattagttcatagcccatatatggagttccgcgttacataacttacggtaaatggcccgcctggctgaccgcccaacgacccccgcccattgacgtcaataatgacgtatgttcccatagtaacgccaatagggactttccattgacgtcaatgggtggagtatttacggtaaactgcccacttggcagtacatcaagtgtatcatatgccaagtacgccccctattgacgtcaatgacggtaaatggcccgcctggcattatgcccagtacatgaccttatgggactttcctacttggcagtacatctacgtattagtcatcgctattaccatggtgatgcggttttggcagtacatcaatgggcgtggatagcggtttgactcacggggatttccaagtctccaccccattgacgtcaatgggagtttgttttggcaccaaaatcaacgggactttccaaaatgtcgtaacaactccgccccattgacgcaaatgggcggtaggcgtgtacggtgggaggtctatataagcagagctcgtttagtgaaccgtcagatcgcctggagacgccatccacgctgttttgacctccatagaagagccaccatgggatggtcatgtatcatcctgttcctagtagcaactgcaaccggtgagatcgtgctgacacagagccctgccacactgtccctgagccctggcgagagagccaccctgagctgtagagccagccagagcgtgagctcctacctggcctggtatcaacagaagcctggccaggctcctagactgctgatctacgatgcctccaatagagccacaggcatcccagccaggttttccggctccggcagcggcaccgatttcaccctgaccatcagcagcctcgaacctgaggatttcgccgtgtactactgtcagcagagatccaattggcctcctagaatcaccttcggccagggcaccaggctggagatcaagggcggcggcggctccggaggaggaggaagcggaggaggcggcagccaggtgcagctggtgcagtccggcgccgaggtgaagaagcctggcgcctccgtgaaggtgagctgcaaggccagcggctacacattcactaggtacaccatgcactgggtcaggcaggctcctggccagggcctggagtggatgggctacatcaacccatccagaggctacaccaactacaatcagaagttcaaggatagagtgaccatcacagccgataagagcaccagcaccgcctacatggagctgtccagcctgagaagcgaggacaccgccgtgtactattgtgccagatactacgatgatcactactgcctggattactggggccagggcacaacagtgacagtgtcctccggcggcggcggaagcggaggcggaggaagcggcggaggaggatctggcagcgagatcgtgctcacacagagccctgctacactgtccctcagccctggcgaaagggccaccctgtcctgtagcgccagcagctccgtgagctacatgaactggtatcaacaaaagcccggcaaggctcctaagaggctgatctacgacacaagcaagctggccagcggcgtgccctccagattctccggctccggaagcggcacagatttcaccctcaccatcaacagcctcgaagccgaggacgccgccacatactactgtcaacagtggtccagcaacccattcacatttggccagggcactaaggtggagatcaagaggggcggcggcgggagcggaggaggaggcagcggaggaggtggcagccaggtccagctgcagcagagcggcgccgaggtcaagaagcctggaagcagcgtgaaggtgtcctgtaaggccagcggaggcacattctcctcctacgccatctcctgggtgagacaggctcctggacagggcctggaatggatgggcggcatcatcccaatcctgggcatcgccaactacgcccagaagttccagggcagagtgacaatcaccgccgacgagtccaccagcacagcctacatggaactgtccagcctcaggtccgaggataccgccgtgtattactgtgccagaggcggcagcggctcctaccacatggatgtgtggggcaagggcacaaccgtgaccgtgagcagctga

SEQ ID NO: 320 - protein, 517 aa, synthetic construct
MGWSCIILFLVATATGEIVLTQSPATLSLSPGERATLSCRASQSVSSYLAWYQQKPGQAPRLLIYDASNRATGIPARFSGSGSGTDFTLTISSLEPEDFAVYYCQQRSNWPPRITFGQGTRLEIKGGGGSGGGGSGGGGSQVQLVQSGAEVKKPGASVKVSCKASGYTFTRYTMHWVRQAPGQGLEWMGYINPSRGYTNYNQKFKDRVTITADKSTSTAYMELSSLRSEDTAVYYCARYYDDHYCLDYWGQGTTVTVSSGGGGSGGGGSGGGGSGSEIVLTQSPATLSLSPGERATLSCSASSSVSYMNWYQQKPGKAPKRLIYDTSKLASGVPSRFSGSGSGTDFTLTINSLEAEDAATYYCQQWSSNPFTFGQGTKVEIKRGGGGSGGGGSGGGGSQVQLQQSGAEVKKPGSSVKVSCKASGGTFSSYAISWVRQAPGQGLEWMGGIIPILGIANYAQKFQGRVTITADESTSTAYMELSSLRSEDTAVYYCARGGSGSYHMDVWGKGTTVTVSS

SEQ ID NO: 321 - DNA, 2207 bp, synthetic construct
  source 1..2207: mol_type = other DNA
gacattgattattgactagttattaatagtaatcaattacggggtcattagttcatagcccatatatggagttccgcgttacataacttacggtaaatggcccgcctggctgaccgcccaacgacccccgcccattgacgtcaataatgacgtatgttcccatagtaacgccaatagggactttccattgacgtcaatgggtggagtatttacggtaaactgcccacttggcagtacatcaagtgtatcatatgccaagtacgccccctattgacgtcaatgacggtaaatggcccgcctggcattatgcccagtacatgaccttatgggactttcctacttggcagtacatctacgtattagtcatcgctattaccatggtgatgcggttttggcagtacatcaatgggcgtggatagcggtttgactcacggggatttccaagtctccaccccattgacgtcaatgggagtttgttttggcaccaaaatcaacgggactttccaaaatgtcgtaacaactccgccccattgacgcaaatgggcggtaggcgtgtacggtgggaggtctatataagcagagctcgtttagtgaaccgtcagatcgcctggagacgccatccacgctgttttgacctccatagaagagccaccatgggatggtcatgtatcatcctgttcctagtagcaactgcaaccggtgatatcgtgatgacccagagccccagcagcctgtctacctctattggcgacagagtgaccattacctgcagagcctcccagggcatcagcaactttctggcctggtttcagcagaagcccggcaaggctcccaagtcactgatctacgccgcctccaggctgcagagtggagtgccttctaaattttccggctccggctctggcaccaacttcactctgactatcagctccctgcagcccgaagacttcgccacatactactgccagcagtacgactcctaccccctgaccttcggcggaggaacaaaggtggagatcaaaggcggcggcggctccggaggaggaggaagcggaggaggcggcagccaggtgcagctggtgcagtccggcgccgaggtgaagaagcctggcgcctccgtgaaggtgagctgcaaggccagcggctacacattcactaggtacaccatgcactgggtcaggcaggctcctggccagggcctggagtggatgggctacatcaacccatccagaggctacaccaactacaatcagaagttcaaggatagagtgaccatcacagccgataagagcaccagcaccgcctacatggagctgtccagcctgagaagcgaggacaccgccgtgtactattgtgccagatactacgatgatcactactgcctggattactggggccagggcacaacagtgacagtgtcctccggcggcggcggaagcggaggcggaggaagcggcggaggaggatctggcagcgagatcgtgctcacacagagccctgctacactgtccctcagccctggcgaaagggccaccctgtcctgtagcgccagcagctccgtgagctacatgaactggtatcaacaaaagcccggcaaggctcctaagaggctgatctacgacacaagcaagctggccagcggcgtgccctccagattctccggctccggaagcggcacagatttcaccctcaccatcaacagcctcgaagccgaggacgccgccacatactactgtcaacagtggtccagcaacccattcacatttggccagggcactaaggtggagatcaagaggggcggcggcgggagcggaggaggaggcagcggaggaggtggcagcgaagtgcagctggtggagagcggaggaggagtggtgcagcctggaagaagcctgacactgagctgcgccgctagcggatttacctttaacggctatagcatgcactgggtgagacaggcccctggaaagggactggagtgggtggctgtgatgagcagcgatggaggaaacaagtactacgctgattccgtgaagggcagattcaccattagccgggacaacagcaagaacacactgtatctgcagatgaacggactgagacccgaggacaccgccgtgtattattgcgccagggccgtgagcagcggatggtctctgcctttcgacttctggggccacggcacactggtgactgtgtctagctga

SEQ ID NO: 322 - protein, 517 aa, synthetic construct
MGWSCIILFLVATATGDIVMTQSPSSLSTSIGDRVTITCRASQGISNFLAWFQQKPGKAPKSLIYAASRLQSGVPSKFSGSGSGTNFTLTISSLQPEDFATYYCQQYDSYPLTFGGGTKVEIKGGGGSGGGGSGGGGSQVQLVQSGAEVKKPGASVKVSCKASGYTFTRYTMHWVRQAPGQGLEWMGYINPSRGYTNYNQKFKDRVTITADKSTSTAYMELSSLRSEDTAVYYCARYYDDHYCLDYWGQGTTVTVSSGGGGSGGGGSGGGGSGSEIVLTQSPATLSLSPGERATLSCSASSSVSYMNWYQQKPGKAPKRLIYDTSKLASGVPSRFSGSGSGTDFTLTINSLEAEDAATYYCQQWSSNPFTFGQGTKVEIKRGGGGSGGGGSGGGGSEVQLVESGGGVVQPGRSLTLSCAASGFTFNGYSMHWVRQAPGKGLEWVAVMSSDGGNKYYADSVKGRFTISRDNSKNTLYLQMNGLRPEDTAVYYCARAVSSGWSLPFDFWGHGTLVTVSS

SEQ ID NO: 323 - DNA, 1616 bp, synthetic construct
  source 1..1616: mol_type = other DNA
atttagaatatatgtatgtaaaaatatagtagaatttcattttgtttttttctatgctataaatgggatggtcatgtatcatcctgttcctagtagcaactgcaaccggtgagatcgtgctgacacagagccctgccacactgtccctgagccctggcgagagagccaccctgagctgtagagccagccagagcgtgagctcctacctggcctggtatcaacagaagcctggccaggctcctagactgctgatctacgatgcctccaatagagccacaggcatcccagccaggttttccggctccggcagcggcaccgatttcaccctgaccatcagcagcctcgaacctgaggatttcgccgtgtactactgtcagcagagatccaattggcctcctagaatcaccttcggccagggcaccaggctggagatcaagggcggcggcggctccggaggaggaggaagcggaggaggcggcagccaggtgcagctggtgcagtccggcgccgaggtgaagaagcctggcgcctccgtgaaggtgagctgcaaggccagcggctacacattcactaggtacaccatgcactgggtcaggcaggctcctggccagggcctggagtggatgggctacatcaacccatccagaggctacaccaactacaatcagaagttcaaggatagagtgaccatcacagccgataagagcaccagcaccgcctacatggagctgtccagcctgagaagcgaggacaccgccgtgtactattgtgccagatactacgatgatcactactgcctggattactggggccagggcacaacagtgacagtgtcctccggcggcggcggaagcggaggcggaggaagcggcggaggaggatctggcagcgagatcgtgctcacacagagccctgctacactgtccctcagccctggcgaaagggccaccctgtcctgtagcgccagcagctccgtgagctacatgaactggtatcaacaaaagcccggcaaggctcctaagaggctgatctacgacacaagcaagctggccagcggcgtgccctccagattctccggctccggaagcggcacagatttcaccctcaccatcaacagcctcgaagccgaggacgccgccacatactactgtcaacagtggtccagcaacccattcacatttggccagggcactaaggtggagatcaagaggggcggcggcgggagcggaggaggaggcagcggaggaggtggcagccaggtccagctgcagcagagcggcgccgaggtcaagaagcctggaagcagcgtgaaggtgtcctgtaaggccagcggaggcacattctcctcctacgccatctcctgggtgagacaggctcctggacagggcctggaatggatgggcggcatcatcccaatcctgggcatcgccaactacgcccagaagttccagggcagagtgacaatcaccgccgacgagtccaccagcacagcctacatggaactgtccagcctcaggtccgaggataccgccgtgtattactgtgccagaggcggcagcggctcctaccacatggatgtgtggggcaagggcacaaccgtgaccgtgagcagctga

SEQ ID NO: 324 - protein, 517 aa, synthetic construct; identical to SEQ ID NO: 320

SEQ ID NO: 325 - DNA, 1616 bp, synthetic construct
  source 1..1616: mol_type = other DNA
atttagaatatatgtatgtaaaaatatagtagaatttcattttgtttttttctatgctataaatgggatggtcatgtatcatcctgttcctagtagcaactgcaaccggtgatatcgtgatgacccagagccccagcagcctgtctacctctattggcgacagagtgaccattacctgcagagcctcccagggcatcagcaactttctggcctggtttcagcagaagcccggcaaggctcccaagtcactgatctacgccgcctccaggctgcagagtggagtgccttctaaattttccggctccggctctggcaccaacttcactctgactatcagctccctgcagcccgaagacttcgccacatactactgccagcagtacgactcctaccccctgaccttcggcggaggaacaaaggtggagatcaaaggcggcggcggctccggaggaggaggaagcggaggaggcggcagccaggtgcagctggtgcagtccggcgccgaggtgaagaagcctggcgcctccgtgaaggtgagctgcaaggccagcggctacacattcactaggtacaccatgcactgggtcaggcaggctcctggccagggcctggagtggatgggctacatcaacccatccagaggctacaccaactacaatcagaagttcaaggatagagtgaccatcacagccgataagagcaccagcaccgcctacatggagctgtccagcctgagaagcgaggacaccgccgtgtactattgtgccagatactacgatgatcactactgcctggattactggggccagggcacaacagtgacagtgtcctccggcggcggcggaagcggaggcggaggaagcggcggaggaggatctggcagcgagatcgtgctcacacagagccctgctacactgtccctcagccctggcgaaagggccaccctgtcctgtagcgccagcagctccgtgagctacatgaactggtatcaacaaaagcccggcaaggctcctaagaggctgatctacgacacaagcaagctggccagcggcgtgccctccagattctccggctccggaagcggcacagatttcaccctcaccatcaacagcctcgaagccgaggacgccgccacatactactgtcaacagtggtccagcaacccattcacatttggccagggcactaaggtggagatcaagaggggcggcggcgggagcggaggaggaggcagcggaggaggtggcagcgaagtgcagctggtggagagcggaggaggagtggtgcagcctggaagaagcctgacactgagctgcgccgctagcggatttacctttaacggctatagcatgcactgggtgagacaggcccctggaaagggactggagtgggtggctgtgatgagcagcgatggaggaaacaagtactacgctgattccgtgaagggcagattcaccattagccgggacaacagcaagaacacactgtatctgcagatgaacggactgagacccgaggacaccgccgtgtattattgcgccagggccgtgagcagcggatggtctctgcctttcgacttctggggccacggcacactggtgactgtgtctagctga

SEQ ID NO: 326 - protein, 517 aa, synthetic construct; identical to SEQ ID NO: 322

SEQ ID NO: 327 - DNA, 2746 bp, synthetic construct
  source 1..2746: mol_type = other DNA
ggctccggtgcccgtcagtgggcagagcgcacatcgcccacagtccccgagaagttggggggaggggtcggcaattgaaccggtgcctagagaaggtggcgcggggtaaactgggaaagtgatgtcgtgtactggctccgcctttttcccgagggtgggggagaaccgtatataagtgcagtagtcgccgtgaacgttctttttcgcaacgggtttgccgccagaacacaggtaagtgccgtgtgtggttcccgcgggcctggcctctttacgggttatggcccttgcgtgccttgaattacttccacctggctccagtacgtgattcttgatcccgagctggagccaggggcgggccttgcgctttaggagccccttcgcctcgtgcttgagttgaggcctggcctgggcgctggggccgccgcgtgcgaatctggtggcaccttcgcgcctgtctcgctgctttcgataagtctctagccatttaaaatttttgatgacctgctgcgacgctttttttctggcaagatagtcttgtaaatgcgggccaggatctgcacactggtatttcggtttttggggccgcgggcggcgacggggcccgtgcgtcccagcgcacatgttcggcgaggcggggcctgcgagcgcggccaccgagaatcggacgggggtcggacgggggtagtctcaagctggccggcctgctctggtgcctggcctcgcgccgccgtgtatcgccccgccctgggcggcaaggctggcccggtcggcaccagttgcgtgagcggaaagatggccgcttcccggccctgctccagggggctcaaaatggaggacgcggcgctcgggagagcgggcgggtgagtcacccacacaaaggaaaggggcctttccgtcctcagccgtcgcttcatgtgactccacggagtaccgggcgccgtccaggcacctcgattagttctggagcttttggagtacgtcgtctttaggttggggggaggggttttatgcgatggagtttccccacactgagtgggtggagactgaagttaggccagcttggcacttgatgtaattctccttggaatttgccctttttgagtttggatcttggttcattctcaagcctcagacagtggttcaaagtttttttcttccatttcaggtgtcgtgacgtttagtgaaccgtcagatcgcctggagacgccatccacgctgttttgacctccatagaagagccaccatggccctgccggtgactgcgttactgttgcccctggccttgctgctgcacgcagcaaggccaggggattacaaagatgacgatgacaaaggatccgagatcgtgctgacacagagccctgccacactgtccctgagccctggcgagagagccaccctgagctgtagagccagccagagcgtgagctcctacctggcctggtatcaacagaagcctggccaggctcctagactgctgatctacgatgcctccaatagagccacaggcatcccagccaggttttccggctccggcagcggcaccgatttcaccctgaccatcagcagcctcgaacctgaggatttcgccgtgtactactgtcagcagagatccaattggcctcctagaatcaccttcggccagggcaccaggctggagatcaagggcggcggcgggagcggaggaggaggcagcggaggaggtggcagccaggtccagctgcagcagagcggcgccgaggtcaagaagcctggaagcagcgtgaaggtgtcctgtaaggccagcggaggcacattctcctcctacgccatctcctgggtgagacaggctcctggacagggcctggaatggatgggcggcatcatcccaatcctgggcatcgccaactacgcccagaagttccagggcagagtgacaatcaccgccgacgagtccaccagcacagcctacatggaactgtccagcctcaggtccgaggataccgccgtgtattactgtgccagaggcggcagcggctcctaccacatggatgtgtggggcaagggcacaaccgtgaccgtgagcagcacgcgtacaactacacccgctcctagacctccaactcctgctcctacaatcgccagccagcctctgtctctgaggccagaagcttgtagacctgctgctggcggagccgtgcatacaagaggactggatttcgcctgcgacatctacatctgggcccctctggctggaacatgtggcgttctgctgctgagcctggtcatcaccctgtactgcaagcggggcagaaagaagctgctgtacatcttcaagcagcccttcatgcggcccgtgcagaccacacaagaggaagatggctgctcctgcagattccccgaggaagaagaaggcggctgcgagctgagagtgaagttcagcagatccgccgacgctcccgcctataagcagggacagaaccagctgtacaacgagctgaacctggggagaagagaagagtacgacgtgctggacaagcggagaggcagagatcctgagatgggcggcaagcccagacggaagaatcctcaagagggcctgtataatgagctgcagaaagacaagatggccgaggcctacagcgagatcggaatgaagggcgagcgcagaagaggcaagggacacgatggactgtaccagggcctgagcaccgccaccaaggatacctatgatgccctgcacatgcaggccctccctcctcgttga

SEQ ID NO: 328 - protein, 500 aa, synthetic construct
MALPVTALLLPLALLLHAARPGDYKDDDDKGSEIVLTQSPATLSLSPGERATLSCRASQSVSSYLAWYQQKPGQAPRLLIYDASNRATGIPARFSGSGSGTDFTLTISSLEPEDFAVYYCQQRSNWPPRITFGQGTRLEIKGGGGSGGGGSGGGGSQVQLQQSGAEVKKPGSSVKVSCKASGGTFSSYAISWVRQAPGQGLEWMGGIIPILGIANYAQKFQGRVTITADESTSTAYMELSSLRSEDTAVYYCARGGSGSYHMDVWGKGTTVTVSSTRTTTPAPRPPTPAPTIASQPLSLRPEACRPAAGGAVHTRGLDFACDIYIWAPLAGTCGVLLLSLVITLYCKRGRKKLLYIFKQPFMRPVQTTQEEDGCSCRFPEEEEGGCELRVKFSRSADAPAYKQGQNQLYNELNLGRREEYDVLDKRRGRDPEMGGKPRRKNPQEGLYNELQKDKMAEAYSEIGMKGERRRGKGHDGLYQGLSTATKDTYDALHMQALPPR

SEQ ID NO: 329 - DNA, 2746 bp, synthetic construct
  source 1..2746: mol_type = other DNA
ggctccggtgcccgtcagtgggcagagcgcacatcgcccacagtccccgagaagttggggggaggggtcggcaattgaaccggtgcctagagaaggtggcgcggggtaaactgggaaagtgatgtcgtgtactggctccgcctttttcccgagggtgggggagaaccgtatataagtgcagtagtcgccgtgaacgttctttttcgcaacgggtttgccgccagaacacaggtaagtgccgtgtgtggttcccgcgggcctggcctctttacgggttatggcccttgcgtgccttgaattacttccacctggctccagtacgtgattcttgatcccgagctggagccaggggcgggccttgcgctttaggagccccttcgcctcgtgcttgagttgaggcctggcctgggcgctggggccgccgcgtgcgaatctggtggcaccttcgcgcctgtctcgctgctttcgataagtctctagccatttaaaatttttgatgacctgctgcgacgctttttttctggcaagatagtcttgtaaatgcgggccaggatctgcacactggtatttcggtttttggggccgcgggcggcgacggggcccgtgcgtcccagcgcacatgttcggcgaggcggggcctgcgagcgcggccaccgagaatcggacgggggtcggacgggggtagtctcaagctggccggcctgctctggtgcctggcctcgcgccgccgtgtatcgccccgccctgggcggcaaggctggcccggtcggcaccagttgcgtgagcggaaagatggccgcttcccggccctgctccagggggctcaaaatggaggacgcggcgctcgggagagcgggcgggtgagtcacccacacaaaggaaaggggcctttccgtcctcagccgtcgcttcatgtgactccacggagtaccgggcgccgtccaggcacctcgattagttctggagcttttggagtacgtcgtctttaggttggggggaggggttttatgcgatggagtttccccacactgagtgggtggagactgaagttaggccagcttggcacttgatgtaattctccttggaatttgccctttttgagtttggatcttggttcattctcaagcctcagacagtggttcaaagtttttttcttccatttcaggtgtcgtgacgtttagtgaaccgtcagatcgcctggagacgccatccacgctgttttgacctccatagaagagccaccatggccctgccggtgactgcgttactgttgcccctggccttgctgctgcacgcagcaaggccaggggattacaaagatgacgatgacaaaggatccgaagtgcagctggtggagagcggaggaggagtggtgcagcctggaagaagcctgacactgagctgcgccgctagcggatttacctttaacggctatagcatgcactgggtgagacaggcccctggaaagggactggagtgggtggctgtgatgagcagcgatggaggaaacaagtactacgctgattccgtgaagggcagattcaccattagccgggacaacagcaagaacacactgtatctgcagatgaacggactgagacccgaggacaccgccgtgtattattgcgccagggccgtgagcagcggatggtctctgcctttcgacttctggggccacggcacactggtgactgtgtctagcggcggaggcggcagcggaggaggaggatctggaggaggaggctctgatatcgtgatgacccagagccccagcagcctgtctacctctattggcgacagagtgaccattacctgcagagcctcccagggcatcagcaactttctggcctggtttcagcagaagcccggcaaggctcccaagtcactgatctacgccgcctccaggctgcagagtggagtgccttctaaattttccggctccggctctggcaccaacttcactctgactatcagctccctgcagcccgaagacttcgccacatactactgccagcagtacgactcctaccccctgaccttcggcggaggaacaaaggtggagatcaaaacgcgtacaactacacccgctcctagacctccaactcctgctcctacaatcgccagccagcctctgtctctgaggccagaagcttgtagacctgctgctggcggagccgtgcatacaagaggactggatttcgcctgcgacatctacatctgggcccctctggctggaacatgtggcgttctgctgctgagcctggtcatcaccctgtactgcaagcggggcagaaagaagctgctgtacatcttcaagcagcccttcatgcggcccgtgcagaccacacaagaggaagatggctgctcctgcagattccccgaggaagaagaaggcggctgcgagctgagagtgaagttcagcagatccgccgacgctcccgcctataagcagggacagaaccagctgtacaacgagctgaacctggggagaagagaagagtacgacgtgctggacaagcggagaggcagagatcctgagatgggcggcaagcccagacggaagaatcctcaagagggcctgtataatgagctgcagaaagacaagatggccgaggcctacagcgagatcggaatgaagggcgagcgcagaagaggcaagggacacgatggactgtaccagggcctgagcaccgccaccaaggatacctatgatgccctgcacatgcaggccctccctcctcgttga

SEQ ID NO: 330 - protein, 500 aa, synthetic construct
MALPVTALLLPLALLLHAARPGDYKDDDDKGSEVQLVESGGGVVQPGRSLTLSCAASGFTFNGYSMHWVRQAPGKGLEWVAVMSSDGGNKYYADSVKGRFTISRDNSKNTLYLQMNGLRPEDTAVYYCARAVSSGWSLPFDFWGHGTLVTVSSGGGGSGGGGSGGGGSDIVMTQSPSSLSTSIGDRVTITCRASQGISNFLAWFQQKPGKAPKSLIYAASRLQSGVPSKFSGSGSGTNFTLTISSLQPEDFATYYCQQYDSYPLTFGGGTKVEIKTRTTTPAPRPPTPAPTIASQPLSLRPEACRPAAGGAVHTRGLDFACDIYIWAPLAGTCGVLLLSLVITLYCKRGRKKLLYIFKQPFMRPVQTTQEEDGCSCRFPEEEEGGCELRVKFSRSADAPAYKQGQNQLYNELNLGRREEYDVLDKRRGRDPEMGGKPRRKNPQEGLYNELQKDKMAEAYSEIGMKGERRRGKGHDGLYQGLSTATKDTYDALHMQALPPR